European Patent Specification EP 3 898 981 B1, published October 18, 2023. Title: METHODS AND COMPOSITIONS FOR TREATING GLYCOGEN STORAGE DISEASES. Applicant: ULTRAGENYX PHARMACEUTICAL INC. The sequence listing filed with the application follows.

SEQUENCE LISTING (15 sequences)

SEQ ID NO: 1 - DNA, 3882 bp, Artificial Sequence
  Description of artificial sequence: DTC177: ITR to ITR
ttggccactccctctctgcgcgctcgctcgctcactgaggccgggcgaccaaaggtcgcccgacgcccgggctttgcccgggcggcctcagtgagcgagcgagcgcgcagagagggagtggccaactccatcactaggggttcctcctttgagaatccacggtgtctcgatgcagtcagctttctaacaagctggggcctcacctgttttcccacggataaaaacgtgctggaggaagcagaaaggggctggcaggtggaaagatgaggaccagctcatcgtctcatgactatgaggttgctctgatccagagggtccccctgcctggtggcccaccgccaggaagactcccactgtccctggatgcccagagtgggatgtcaactccatcacttatcaactccttatccataggggtattcttcctgaggcgtctcagaaaacagggccctccccatatgctgaccacataatagaacccctcccaactcagagaccctggctgctagctgccctggcatgacccagacagtggcctttgtatatgtttttagactcaccttgactcacctctgaccatagaaactctcatcccagaggtcactgcaatagttactccacaacagaggcttatctgggtagagggaggctccctacctatggcccagcagccctgacagtgcagatcacatataccccacgccccagcactgcctgccacgcatgggcttactttacacccacccacagtcaccaacacattacctgctctccaaggttaggcgtggcaggagaagtttgcttggaccagcagaaaccatgcagtcaaggacaactggagtcagcatgggctgggtgcgagcccttggtggggtggggaggagactccaggtcatacctcctggaggatgttttaatcatttccagcatggaatgctgtcaacttttgccacagattcattagctctgagtttcttttttctgtccccagctaccccttacatgtcaatatggacttaatgatgggaaattcaggcaagtttttaaacattttattccccctggctcttatcctcaaaaaatgcatgagttcgttacctgattcattccctggttcctttcacagtcctccgtgacccaagtgttagggttttggtctctctactatttgtaggctgatatatagtatacacacacacacacacacacatatacacacacacagtgtatcttgagctttcttttgtatatctacacacatatgtataagaaagctcaagatatagaagccctttttcaaaaataactgaaagtttcaaactctttaagtctccagttaccattttgctggtattcttatttggaaccatacattcatcatattgttgcacagtaagactatacattcattattttgcttaaacgtatgagttaaaacactttaaggtcattaaatgaattaatcactgcattcaaaaacgattactttctggccctaagagacatgaggccaataccaggaagggggttgatctcccaaaccagaggcagaccctagactctaatacagttaaggaaagaccagcaagatgatagtccccaatacaatagaactttactaattttaaaattaagaacttaaaacttgaatagctagagcaccaagatttttctttgtccccaaataagtgcagttgcaggcatagaaaatctgacatctttgcaagaatcatcgtggatgtagactctgtcctgtgtctctggcctggtttcggggaccaggagggcagacccttgcactgccaagaagcatgccaaagttaatcattggccctgctgagtacatggccgatcaggctgtttttgtgtgcctgtttttctattttacgtaaatcaccctgaacatgtttgcatcaacctactggtgatgcacctttgatcaatacattttagacaaacgtggtttttgagtccaaagatcagggctgggttgacctgaatactggatacagggcatataaaacaggggcaaggcacagactcatagcagagcaatcaccaccaagcctggaataactgcaagggctctgctgacatcttcctgaggtgccaaggaaatgaggtctagagaagctttattgcggtagtttatcacagttaaattgctaacgcagtcagtgcttctgacacaacagtctcgaacttaagctgcagtgactctcttaaggtagccttgcagaagttggtcgtgaggcactgggcaggtaagtatcaaggttacaagacaggtttaaggagaccaatagaaactgggcttgtcgagacagagaagactcttgcgtttctgataggcacctattggtcttactgacatccactttgcctttctctccacaggtgtccactcccagttcaattacagctcttaaggccctgcaggccaccatggaagagggcatgaacgtgctgcacgacttcggcatccagagcacccactatctgcaggtcaactaccaggacagccaggactggttcatcctggtgtccgtgatcgccgacctgcggaacgccttctacgtgctgttccccatctggttccatctgcaagaagccgtcggcatcaagctgctgtgggtggccgtgatcggcgattggctgaacctggtgttcaagtggatcctgttcggccagcggccctattggtgggtgctggacaccgactactacagcaacaccagcgtgcccctgatcaagcagttccccgtgacctgcgagacaggccctggctctccttctggccacgccatgggaacagccggcgtgtactacgtgatggtcaccagcaccctgagcatcttccagggcaagatcaagcccacctaccggttccggtgcctgaacgtgatcctgtggctgggcttctgggccgtgcagctgaacgtgtgcctgagccggatctacctggccgcccacttcccacatcaagtggtggccggcgtgctgagcggaatcgccgtggccgagacattcagccacatccacagcatctacaacgccagcctgaagaagtacttcctgatcacattctttctgttcagcttcgccatcggcttctacctgctgctgaagggcctgggcgtggacctgctgtggaccctggaaaaggcccagcggtggtgcgagcagcccgagtgggtgcacatcgacaccacccccttcgccagcctgctgaagaacctgggcaccctgtttggactgggcctggccctgaacagcagcatgtacagagagagctgcaagggcaagctgagcaagtggctgcccttccggctgagcagcatcgtggccagcctggtgctgctgcacgtgttcgacagcctgaagccccccagccaggtggaactggtgttttacgtgctgagcttctgcaagagcgccgtggtgcccctggcctccgtgtctgtgatcccctactgcctggctcaggtgctgggccagccccacaagaagtccctctgagcgctctaggcggccgcgcggatccagacatgataagatacattgatgagtttggacaaaccacaactagaatgcagtgaaaaaaatgctttatttgtgaaatttgtgatgctattgctttatttgtaaccattataagctgcaataaacaagttaacaacaacaattgcattcattttatgtttcaggttcagggggaggtgtgggaggttttttagaggaacccctagtgatggagttggccactccctctctgcgcgctcgctcgctcactgaggccgcccgggcaaagcccgggcgtcgggcgacctttggtcgcccggcctcagtgagcgagcgagcgcgcagagagggagtggccaa

SEQ ID NO: 2 - DNA, 3882 bp, Artificial Sequence
  Description of artificial sequence: DTC177wt: Replacement of coG6PC sequence with wildtype coding sequence
ttggccactccctctctgcgcgctcgctcgctcactgaggccgggcgaccaaaggtcgcccgacgcccgggctttgcccgggcggcctcagtgagcgagcgagcgcgcagagagggagtggccaactccatcactaggggttcctcctttgagaatccacggtgtctcgatgcagtcagctttctaacaagctggggcctcacctgttttcccacggataaaaacgtgctggaggaagcagaaaggggctggcaggtggaaagatgaggaccagctcatcgtctcatgactatgaggttgctctgatccagagggtccccctgcctggtggcccaccgccaggaagactcccactgtccctggatgcccagagtgggatgtcaactccatcacttatcaactccttatccataggggtattcttcctgaggcgtctcagaaaacagggccctccccatatgctgaccacataatagaacccctcccaactcagagaccctggctgctagctgccctggcatgacccagacagtggcctttgtatatgtttttagactcaccttgactcacctctgaccatagaaactctcatcccagaggtcactgcaatagttactccacaacagaggcttatctgggtagagggaggctccctacctatggcccagcagccctgacagtgcagatcacatataccccacgccccagcactgcctgccacgcatgggcttactttacacccacccacagtcaccaacacattacctgctctccaaggttaggcgtggcaggagaagtttgcttggaccagcagaaaccatgcagtcaaggacaactggagtcagcatgggctgggtgcgagcccttggtggggtggggaggagactccaggtcatacctcctggaggatgttttaatcatttccagcatggaatgctgtcaacttttgccacagattcattagctctgagtttcttttttctgtccccagctaccccttacatgtcaatatggacttaatgatgggaaattcaggcaagtttttaaacattttattccccctggctcttatcctcaaaaaatgcatgagttcgttacctgattcattccctggttcctttcacagtcctccgtgacccaagtgttagggttttggtctctctactatttgtaggctgatatatagtatacacacacacacacacacacatatacacacacacagtgtatcttgagctttcttttgtatatctacacacatatgtataagaaagctcaagatatagaagccctttttcaaaaataactgaaagtttcaaactctttaagtctccagttaccattttgctggtattcttatttggaaccatacattcatcatattgttgcacagtaagactatacattcattattttgcttaaacgtatgagttaaaacactttaaggtcattaaatgaattaatcactgcattcaaaaacgattactttctggccctaagagacatgaggccaataccaggaagggggttgatctcccaaaccagaggcagaccctagactctaatacagttaaggaaagaccagcaagatgatagtccccaatacaatagaactttactaattttaaaattaagaacttaaaacttgaatagctagagcaccaagatttttctttgtccccaaataagtgcagttgcaggcatagaaaatctgacatctttgcaagaatcatcgtggatgtagactctgtcctgtgtctctggcctggtttcggggaccaggagggcagacccttgcactgccaagaagcatgccaaagttaatcattggccctgctgagtacatggccgatcaggctgtttttgtgtgcctgtttttctattttacgtaaatcaccctgaacatgtttgcatcaacctactggtgatgcacctttgatcaatacattttagacaaacgtggtttttgagtccaaagatcagggctgggttgacctgaatactggatacagggcatataaaacaggggcaaggcacagactcatagcagagcaatcaccaccaagcctggaataactgcaagggctctgctgacatcttcctgaggtgccaaggaaatgaggtctagagaagctttattgcggtagtttatcacagttaaattgctaacgcagtcagtgcttctgacacaacagtctcgaacttaagctgcagtgactctcttaaggtagccttgcagaagttggtcgtgaggcactgggcaggtaagtatcaaggttacaagacaggtttaaggagaccaatagaaactgggcttgtcgagacagagaagactcttgcgtttctgataggcacctattggtcttactgacatccactttgcctttctctccacaggtgtccactcccagttcaattacagctcttaaggccctgcaggccaccatggaggaaggaatgaatgttctccatgactttgggatccagtcaacacattacctccaggtgaattaccaagactcccaggactggttcatcttggtgtccgtgatcgcagacctcaggaatgccttctacgtcctcttccccatctggttccatcttcaggaagctgtgggcattaaactcctttgggtagctgtgattggagactggctcaacctcgtctttaagtggattctctttggacagcgtccatactggtgggttttggatactgactactacagcaacacttccgtgcccctgataaagcagttccctgtaacctgtgagactggaccagggagcccctctggccatgccatgggcacagcaggtgtatactacgtgatggtcacatctactctttccatctttcagggaaagataaagccgacctacagatttcggtgcttgaatgtcattttgtggttgggattctgggctgtgcagctgaatgtctgtctgtcacgaatctaccttgctgctcattttcctcatcaagttgttgctggagtcctgtcaggcattgctgttgcagaaactttcagccacatccacagcatctataatgccagcctcaagaaatattttctcattaccttcttcctgttcagcttcgccatcggattttatctgctgctcaagggactgggtgtagacctcctgtggactctggagaaagcccagaggtggtgcgagcagccagaatgggtccacattgacaccacaccctttgccagcctcctcaagaacctgggcacgctctttggcctggggctggctctcaactccagcatgtacagggagagctgcaaggggaaactcagcaagtggctcccattccgcctcagctctattgtagcctccctcgtcctcctgcacgtctttgactccttgaaacccccatcccaagtcgagctggtcttctacgtcttgtccttctgcaagagtgcggtagtgcccctggcatccgtcagtgtcatcccctactgcctcgcccaggtcctgggccagccgcacaagaagtcgttgtaagcgctctaggcggccgcgcggatccagacatgataagatacattgatgagtttggacaaaccacaactagaatgcagtgaaaaaaatgctttatttgtgaaatttgtgatgctattgctttatttgtaaccattataagctgcaataaacaagttaacaacaacaattgcattcattttatgtttcaggttcagggggaggtgtgggaggttttttagaggaacccctagtgatggagttggccactccctctctgcgcgctcgctcgctcactgaggccgcccgggcaaagcccgggcgtcgggcgacctttggtcgcccggcctcagtgagcgagcgagcgcgcagagagggagtggccaa

SEQ ID NO: 3 - DNA, 1074 bp, Artificial Sequence
  Description of Artificial Sequence: Codon-optimized G6PC coding sequence
atggaagagggcatgaacgtgctgcacgacttcggcatccagagcacccactatctgcaggtcaactaccaggacagccaggactggttcatcctggtgtccgtgatcgccgacctgcggaacgccttctacgtgctgttccccatctggttccatctgcaagaagccgtcggcatcaagctgctgtgggtggccgtgatcggcgattggctgaacctggtgttcaagtggatcctgttcggccagcggccctattggtgggtgctggacaccgactactacagcaacaccagcgtgcccctgatcaagcagttccccgtgacctgcgagacaggccctggctctccttctggccacgccatgggaacagccggcgtgtactacgtgatggtcaccagcaccctgagcatcttccagggcaagatcaagcccacctaccggttccggtgcctgaacgtgatcctgtggctgggcttctgggccgtgcagctgaacgtgtgcctgagccggatctacctggccgcccacttcccacatcaagtggtggccggcgtgctgagcggaatcgccgtggccgagacattcagccacatccacagcatctacaacgccagcctgaagaagtacttcctgatcacattctttctgttcagcttcgccatcggcttctacctgctgctgaagggcctgggcgtggacctgctgtggaccctggaaaaggcccagcggtggtgcgagcagcccgagtgggtgcacatcgacaccacccccttcgccagcctgctgaagaacctgggcaccctgtttggactgggcctggccctgaacagcagcatgtacagagagagctgcaagggcaagctgagcaagtggctgcccttccggctgagcagcatcgtggccagcctggtgctgctgcacgtgttcgacagcctgaagccccccagccaggtggaactggtgttttacgtgctgagcttctgcaagagcgccgtggtgcccctggcctccgtgtctgtgatcccctactgcctggctcaggtgctgggccagccccacaagaagtccctctga

SEQ ID NO: 4 - DNA, 1074 bp, Homo sapiens
atggaggaaggaatgaatgttctccatgactttgggatccagtcaacacattacctccaggtgaattaccaagactcccaggactggttcatcttggtgtccgtgatcgcagacctcaggaatgccttctacgtcctcttccccatctggttccatcttcaggaagctgtgggcattaaactcctttgggtagctgtgattggagactggctcaacctcgtctttaagtggattctctttggacagcgtccatactggtgggttttggatactgactactacagcaacacttccgtgcccctgataaagcagttccctgtaacctgtgagactggaccagggagcccctctggccatgccatgggcacagcaggtgtatactacgtgatggtcacatctactctttccatctttcagggaaagataaagccgacctacagatttcggtgcttgaatgtcattttgtggttgggattctgggctgtgcagctgaatgtctgtctgtcacgaatctaccttgctgctcattttcctcatcaagttgttgctggagtcctgtcaggcattgctgttgcagaaactttcagccacatccacagcatctataatgccagcctcaagaaatattttctcattaccttcttcctgttcagcttcgccatcggattttatctgctgctcaagggactgggtgtagacctcctgtggactctggagaaagcccagaggtggtgcgagcagccagaatgggtccacattgacaccacaccctttgccagcctcctcaagaacctgggcacgctctttggcctggggctggctctcaactccagcatgtacagggagagctgcaaggggaaactcagcaagtggctcccattccgcctcagctctattgtagcctccctcgtcctcctgcacgtctttgactccttgaaacccccatcccaagtcgagctggtcttctacgtcttgtccttctgcaagagtgcggtagtgcccctggcatccgtcagtgtcatcccctactgcctcgcccaggtcctgggccagccgcacaagaagtcgttgtaa

SEQ ID NO: 5 - protein, 357 aa, Homo sapiens
MEEGMNVLHDFGIQSTHYLQVNYQDSQDWFILVSVIADLRNAFYVLFPIWFHLQEAVGIKLLWVAVIGDWLNLVFKWILFGQRPYWWVLDTDYYSNTSVPLIKQFPVTCETGPGSPSGHAMGTAGVYYVMVTSTLSIFQGKIKPTYRFRCLNVILWLGFWAVQLNVCLSRIYLAAHFPHQVVAGVLSGIAVAETFSHIHSIYNASLKKYFLITFFLFSFAIGFYLLLKGLGVDLLWTLEKAQRWCEQPEWVHIDTTPFASLLKNLGTLFGLGLALNSSMYRESCKGKLSKWLPFRLSSIVASLVLLHVFDSLKPPSQVELVFYVLSFCKSAVVPLASVSVIPYCLAQVLGQPHKKSL

SEQ ID NO: 6 - DNA, 2864 bp, Homo sapiens
cctttgagaatccacggtgtctcgatgcagtcagctttctaacaagctggggcctcacctgttttcccacggataaaaacgtgctggaggaagcagaaaggggctggcaggtggaaagatgaggaccagctcatcgtctcatgactatgaggttgctctgatccagagggtccccctgcctggtggcccaccgccaggaagactcccactgtccctggatgcccagagtgggatgtcaactccatcacttatcaactccttatccataggggtattcttcctgaggcgtctcagaaaacagggccctccccatatgctgaccacataatagaacccctcccaactcagagaccctggctgctagctgccctggcatgacccagacagtggcctttgtatatgtttttagactcaccttgactcacctctgaccatagaaactctcatcccagaggtcactgcaatagttactccacaacagaggcttatctgggtagagggaggctccctacctatggcccagcagccctgacagtgcagatcacatataccccacgccccagcactgcctgccacgcatgggcttactttacacccacccacagtcaccaacacattacctgctctccaaggttaggcgtggcaggagaagtttgcttggaccagcagaaaccatgcagtcaaggacaactggagtcagcatgggctgggtgcgagcccttggtggggtggggaggagactccaggtcatacctcctggaggatgttttaatcatttccagcatggaatgctgtcaacttttgccacagattcattagctctgagtttcttttttctgtccccagctaccccttacatgtcaatatggacttaatgatgggaaattcaggcaagtttttaaacattttattccccctggctcttatcctcaaaaaatgcatgaatttggaggcagtggctcatgcctgtaatcccaatgctttgctaggttgaggcgggaggatcacttgaagccaggaatttgagaccagcctgggccgcatagtgagaccccgtttctacaaaaataaataaataaataataaataatagtgatatgaagcatgattaaatagccctattttttaaaatgcatgagttcgttacctgattcattccctggttcctttcacagtcctccgtgacccaagtgttagggttttggtctctctactatttgtaggctgatatatagtatacacacacacacacacacacatatacacacacacagtgtatcttgagctttcttttgtatatctacacacatatgtataagaaagctcaagatatagaagccctttttcaaaaataactgaaagtttcaaactctttaagtctccagttaccattttgctggtattcttatttggaaccatacattcatcatattgttgcacagtaagactatacattcattattttgcttaaacgtatgagttaaaacacttggccaggcatggtggttcacacctgtaatcccagagctttgggaagccaagactggcagatctcttgagctcaggaattcaagaccagcctgggcaacatggaaaaaccccatctctacaaaagatagaaaaattagccaggcatggtggcgtgtgcctgtggtcccagctactcaggaggctgaggtgggaggatcacattagcccaggaggttgaggctgcagtgagccgtgattatgccactgcactccagcctgggagacagagtgagaccctgtttcaaaaaaaagagagagaaaatttaaaaaagaaaacaacaccaagggctgtaactttaaggtcattaaatgaattaatcactgcattcaaaaacgattactttctggccctaagagacatgaggccaataccaggaagggggttgatctcccaaaccagaggcagaccctagactctaatacagttaaggaaagaccagcaagatgatagtccccaatacaatagaagttactatattttatttgttgtttttcttttgttttgttttgttttgttttgttttgttttagagactggggtcttgctcgattgcccaggctgtagtgcagcggtgggacaatagctcactgcagactccaactcctgggctcaagcaatcctcctgcctcagcctcctgaatagctgggactacaagggtacaccatcacacacaccaaaacaattttttaaatttttgtgtagaaacgagggtcttgctttgttgcccaggctggtctccaactcctggcttcaagggatcctcccacctcagcctcccaaattgctgggattacaggtgtgagccaccacaaccagccagaactttactaattttaaaattaagaacttaaaacttgaatagctagagcaccaagatttttctttgtccccaaataagtgcagttgcaggcatagaaaatctgacatctttgcaagaatcatcgtggatgtagactctgtcctgtgtctctggcctggtttcggggaccaggagggcagacccttgcactgccaagaagcatgccaaagttaatcattggccctgctgagtacatggccgatcaggctgtttttgtgtgcctgtttttctattttacgtaaatcaccctgaacatgtttgcatcaacctactggtgatgcacctttgatcaatacattttagacaaacgtggtttttgagtccaaagatcagggctgggttgacctgaatactggatacagggcatataaaacaggggcaaggcacagactcatagcagagcaatcaccaccaagcctggaataactgcaagggctctgctgacatcttcctgaggtgccaaggaaatgagg

SEQ ID NO: 7 - DNA, 2670 bp, Artificial Sequence
  Description of Artificial Sequence: wildtype GPE but lacking Alu - 1
cctttgagaatccacggtgtctcgatgcagtcagctttctaacaagctggggcctcacctgttttcccacggataaaaacgtgctggaggaagcagaaaggggctggcaggtggaaagatgaggaccagctcatcgtctcatgactatgaggttgctctgatccagagggtccccctgcctggtggcccaccgccaggaagactcccactgtccctggatgcccagagtgggatgtcaactccatcacttatcaactccttatccataggggtattcttcctgaggcgtctcagaaaacagggccctccccatatgctgaccacataatagaacccctcccaactcagagaccctggctgctagctgccctggcatgacccagacagtggcctttgtatatgtttttagactcaccttgactcacctctgaccatagaaactctcatcccagaggtcactgcaatagttactccacaacagaggcttatctgggtagagggaggctccctacctatggcccagcagccctgacagtgcagatcacatataccccacgccccagcactgcctgccacgcatgggcttactttacacccacccacagtcaccaacacattacctgctctccaaggttaggcgtggcaggagaagtttgcttggaccagcagaaaccatgcagtcaaggacaactggagtcagcatgggctgggtgcgagcccttggtggggtggggaggagactccaggtcatacctcctggaggatgttttaatcatttccagcatggaatgctgtcaacttttgccacagattcattagctctgagtttcttttttctgtccccagctaccccttacatgtcaatatggacttaatgatgggaaattcaggcaagtttttaaacattttattccccctggctcttatcctcaaaaaatgcatgagttcgttacctgattcattccctggttcctttcacagtcctccgtgacccaagtgttagggttttggtctctctactatttgtaggctgatatatagtatacacacacacacacacacacatatacacacacacagtgtatcttgagctttcttttgtatatctacacacatatgtataagaaagctcaagatatagaagccctttttcaaaaataactgaaagtttcaaactctttaagtctccagttaccattttgctggtattcttatttggaaccatacattcatcatattgttgcacagtaagactatacattcattattttgcttaaacgtatgagttaaaacacttggccaggcatggtggttcacacctgtaatcccagagctttgggaagccaagactggcagatctcttgagctcaggaattcaagaccagcctgggcaacatggaaaaaccccatctctacaaaagatagaaaaattagccaggcatggtggcgtgtgcctgtggtcccagctactcaggaggctgaggtgggaggatcacattagcccaggaggttgaggctgcagtgagccgtgattatgccactgcactccagcctgggagacagagtgagaccctgtttcaaaaaaaagagagagaaaatttaaaaaagaaaacaacaccaagggctgtaactttaaggtcattaaatgaattaatcactgcattcaaaaacgattactttctggccctaagagacatgaggccaataccaggaagggggttgatctcccaaaccagaggcagaccctagactctaatacagttaaggaaagaccagcaagatgatagtccccaatacaatagaagttactatattttatttgttgtttttcttttgttttgttttgttttgttttgttttgttttagagactggggtcttgctcgattgcccaggctgtagtgcagcggtgggacaatagctcactgcagactccaactcctgggctcaagcaatcctcctgcctcagcctcctgaatagctgggactacaagggtacaccatcacacacaccaaaacaattttttaaatttttgtgtagaaacgagggtcttgctttgttgcccaggctggtctccaactcctggcttcaagggatcctcccacctcagcctcccaaattgctgggattacaggtgtgagccaccacaaccagccagaactttactaattttaaaattaagaacttaaaacttgaatagctagagcaccaagatttttctttgtccccaaataagtgcagttgcaggcatagaaaatctgacatctttgcaagaatcatcgtggatgtagactctgtcctgtgtctctggcctggtttcggggaccaggagggcagacccttgcactgccaagaagcatgccaaagttaatcattggccctgctgagtacatggccgatcaggctgtttttgtgtgcctgtttttctattttacgtaaatcaccctgaacatgtttgcatcaacctactggtgatgcacctttgatcaatacattttagacaaacgtggtttttgagtccaaagatcagggctgggttgacctgaatactggatacagggcatataaaacaggggcaaggcacagactcatagcagagcaatcaccaccaagcctggaataactgcaagggctctgctgacatcttcctgaggtgccaaggaaatgagg

SEQ ID NO: 8 - DNA, 2528 bp, Artificial Sequence
  Description of Artificial Sequence: wildtype GPE but lacking Alu - 2
cctttgagaatccacggtgtctcgatgcagtcagctttctaacaagctggggcctcacctgttttcccacggataaaaacgtgctggaggaagcagaaaggggctggcaggtggaaagatgaggaccagctcatcgtctcatgactatgaggttgctctgatccagagggtccccctgcctggtggcccaccgccaggaagactcccactgtccctggatgcccagagtgggatgtcaactccatcacttatcaactccttatccataggggtattcttcctgaggcgtctcagaaaacagggccctccccatatgctgaccacataatagaacccctcccaactcagagaccctggctgctagctgccctggcatgacccagacagtggcctttgtatatgtttttagactcaccttgactcacctctgaccatagaaactctcatcccagaggtcactgcaatagttactccacaacagaggcttatctgggtagagggaggctccctacctatggcccagcagccctgacagtgcagatcacatataccccacgccccagcactgcctgccacgcatgggcttactttacacccacccacagtcaccaacacattacctgctctccaaggttaggcgtggcaggagaagtttgcttggaccagcagaaaccatgcagtcaaggacaactggagtcagcatgggctgggtgcgagcccttggtggggtggggaggagactccaggtcatacctcctggaggatgttttaatcatttccagcatggaatgctgtcaacttttgccacagattcattagctctgagtttcttttttctgtccccagctaccccttacatgtcaatatggacttaatgatgggaaattcaggcaagtttttaaacattttattccccctggctcttatcctcaaaaaatgcatgaatttggaggcagtggctcatgcctgtaatcccaatgctttgctaggttgaggcgggaggatcacttgaagccaggaatttgagaccagcctgggccgcatagtgagaccccgtttctacaaaaataaataaataaataataaataatagtgatatgaagcatgattaaatagccctattttttaaaatgcatgagttcgttacctgattcattccctggttcctttcacagtcctccgtgacccaagtgttagggttttggtctctctactatttgtaggctgatatatagtatacacacacacacacacacacatatacacacacacagtgtatcttgagctttcttttgtatatctacacacatatgtataagaaagctcaagatatagaagccctttttcaaaaataactgaaagtttcaaactctttaagtctccagttaccattttgctggtattcttatttggaaccatacattcatcatattgttgcacagtaagactatacattcattattttgcttaaacgtatgagttaaaacactttaaggtcattaaatgaattaatcactgcattcaaaaacgattactttctggccctaagagacatgaggccaataccaggaagggggttgatctcccaaaccagaggcagaccctagactctaatacagttaaggaaagaccagcaagatgatagtccccaatacaatagaagttactatattttatttgttgtttttcttttgttttgttttgttttgttttgttttgttttagagactggggtcttgctcgattgcccaggctgtagtgcagcggtgggacaatagctcactgcagactccaactcctgggctcaagcaatcctcctgcctcagcctcctgaatagctgggactacaagggtacaccatcacacacaccaaaacaattttttaaatttttgtgtagaaacgagggtcttgctttgttgcccaggctggtctccaactcctggcttcaagggatcctcccacctcagcctcccaaattgctgggattacaggtgtgagccaccacaaccagccagaactttactaattttaaaattaagaacttaaaacttgaatagctagagcaccaagatttttctttgtccccaaataagtgcagttgcaggcatagaaaatctgacatctttgcaagaatcatcgtggatgtagactctgtcctgtgtctctggcctggtttcggggaccaggagggcagacccttgcactgccaagaagcatgccaaagttaatcattggccctgctgagtacatggccgatcaggctgtttttgtgtgcctgtttttctattttacgtaaatcaccctgaacatgtttgcatcaacctactggtgatgcacctttgatcaatacattttagacaaacgtggtttttgagtccaaagatcagggctgggttgacctgaatactggatacagggcatataaaacaggggcaaggcacagactcatagcagagcaatcaccaccaagcctggaataactgcaagggctctgctgacatcttcctgaggtgccaaggaaatgagg

SEQ ID NO: 9 - DNA, 2508 bp, Artificial Sequence
  Description of Artificial Sequence: wildtype GPE but  lacking Alu - 3
cctttgagaatccacggtgtctcgatgcagtcagctttctaacaagctggggcctcacctgttttcccacggataaaaacgtgctggaggaagcagaaaggggctggcaggtggaaagatgaggaccagctcatcgtctcatgactatgaggttgctctgatccagagggtccccctgcctggtggcccaccgccaggaagactcccactgtccctggatgcccagagtgggatgtcaactccatcacttatcaactccttatccataggggtattcttcctgaggcgtctcagaaaacagggccctccccatatgctgaccacataatagaacccctcccaactcagagaccctggctgctagctgccctggcatgacccagacagtggcctttgtatatgtttttagactcaccttgactcacctctgaccatagaaactctcatcccagaggtcactgcaatagttactccacaacagaggcttatctgggtagagggaggctccctacctatggcccagcagccctgacagtgcagatcacatataccccacgccccagcactgcctgccacgcatgggcttactttacacccacccacagtcaccaacacattacctgctctccaaggttaggcgtggcaggagaagtttgcttggaccagcagaaaccatgcagtcaaggacaactggagtcagcatgggctgggtgcgagcccttggtggggtggggaggagactccaggtcatacctcctggaggatgttttaatcatttccagcatggaatgctgtcaacttttgccacagattcattagctctgagtttcttttttctgtccccagctaccccttacatgtcaatatggacttaatgatgggaaattcaggcaagtttttaaacattttattccccctggctcttatcctcaaaaaatgcatgaatttggaggcagtggctcatgcctgtaatcccaatgctttgctaggttgaggcgggaggatcacttgaagccaggaatttgagaccagcctgggccgcatagtgagaccccgtttctacaaaaataaataaataaataataaataatagtgatatgaagcatgattaaatagccctattttttaaaatgcatgagttcgttacctgattcattccctggttcctttcacagtcctccgtgacccaagtgttagggttttggtctctctactatttgtaggctgatatatagtatacacacacacacacacacacatatacacacacacagtgtatcttgagctttcttttgtatatctacacacatatgtataagaaagctcaagatatagaagccctttttcaaaaataactgaaagtttcaaactctttaagtctccagttaccattttgctggtattcttatttggaaccatacattcatcatattgttgcacagtaagactatacattcattattttgcttaaacgtatgagttaaaacacttggccaggcatggtggttcacacctgtaatcccagagctttgggaagccaagactggcagatctcttgagctcaggaattcaagaccagcctgggcaacatggaaaaaccccatctctacaaaagatagaaaaattagccaggcatggtggcgtgtgcctgtggtcccagctactcaggaggctgaggtgggaggatcacattagcccaggaggttgaggctgcagtgagccgtgattatgccactgcactccagcctgggagacagagtgagaccctgtttcaaaaaaaagagagagaaaatttaaaaaagaaaacaacaccaagggctgtaactttaaggtcattaaatgaattaatcactgcattcaaaaacgattactttctggccctaagagacatgaggccaataccaggaagggggttgatctcccaaaccagaggcagaccctagactctaatacagttaaggaaagaccagcaagatgatagtccccaatacaatagaactttactaattttaaaattaagaacttaaaacttgaatagctagagcaccaagatttttctttgtccccaaataagtgcagttgcaggcatagaaaatctgacatctttgcaagaatcatcgtggatgtagactctgtcctgtgtctctggcctggtttcggggaccaggagggcagacccttgcactgccaagaagcatgccaaagttaatcattggccctgctgagtacatggccgatcaggctgtttttgtgtgcctgtttttctattttacgtaaatcaccctgaacatgtttgcatcaacctactggtgatgcacctttgatcaatacattttagacaaacgtggtttttgagtccaaagatcagggctgggttgacctgaatactggatacagggcatataaaacaggggcaaggcacagactcatagcagagcaatcaccaccaagcctggaataactgcaagggctctgctgacatcttcctgaggtgccaaggaaatgagg

SEQ ID NO: 10 - DNA, 2334 bp, Artificial Sequence
  Description of Artificial Sequence: wildtype GPE, but lacking Alu - 1 and Alu - 2
cctttgagaatccacggtgtctcgatgcagtcagctttctaacaagctggggcctcacctgttttcccacggataaaaacgtgctggaggaagcagaaaggggctggcaggtggaaagatgaggaccagctcatcgtctcatgactatgaggttgctctgatccagagggtccccctgcctggtggcccaccgccaggaagactcccactgtccctggatgcccagagtgggatgtcaactccatcacttatcaactccttatccataggggtattcttcctgaggcgtctcagaaaacagggccctccccatatgctgaccacataatagaacccctcccaactcagagaccctggctgctagctgccctggcatgacccagacagtggcctttgtatatgtttttagactcaccttgactcacctctgaccatagaaactctcatcccagaggtcactgcaatagttactccacaacagaggcttatctgggtagagggaggctccctacctatggcccagcagccctgacagtgcagatcacatataccccacgccccagcactgcctgccacgcatgggcttactttacacccacccacagtcaccaacacattacctgctctccaaggttaggcgtggcaggagaagtttgcttggaccagcagaaaccatgcagtcaaggacaactggagtcagcatgggctgggtgcgagcccttggtggggtggggaggagactccaggtcatacctcctggaggatgttttaatcatttccagcatggaatgctgtcaacttttgccacagattcattagctctgagtttcttttttctgtccccagctaccccttacatgtcaatatggacttaatgatgggaaattcaggcaagtttttaaacattttattccccctggctcttatcctcaaaaaatgcatgagttcgttacctgattcattccctggttcctttcacagtcctccgtgacccaagtgttagggttttggtctctctactatttgtaggctgatatatagtatacacacacacacacacacacatatacacacacacagtgtatcttgagctttcttttgtatatctacacacatatgtataagaaagctcaagatatagaagccctttttcaaaaataactgaaagtttcaaactctttaagtctccagttaccattttgctggtattcttatttggaaccatacattcatcatattgttgcacagtaagactatacattcattattttgcttaaacgtatgagttaaaacactttaaggtcattaaatgaattaatcactgcattcaaaaacgattactttctggccctaagagacatgaggccaataccaggaagggggttgatctcccaaaccagaggcagaccctagactctaatacagttaaggaaagaccagcaagatgatagtccccaatacaatagaagttactatattttatttgttgtttttcttttgttttgttttgttttgttttgttttgttttagagactggggtcttgctcgattgcccaggctgtagtgcagcggtgggacaatagctcactgcagactccaactcctgggctcaagcaatcctcctgcctcagcctcctgaatagctgggactacaagggtacaccatcacacacaccaaaacaattttttaaatttttgtgtagaaacgagggtcttgctttgttgcccaggctggtctccaactcctggcttcaagggatcctcccacctcagcctcccaaattgctgggattacaggtgtgagccaccacaaccagccagaactttactaattttaaaattaagaacttaaaacttgaatagctagagcaccaagatttttctttgtccccaaataagtgcagttgcaggcatagaaaatctgacatctttgcaagaatcatcgtggatgtagactctgtcctgtgtctctggcctggtttcggggaccaggagggcagacccttgcactgccaagaagcatgccaaagttaatcattggccctgctgagtacatggccgatcaggctgtttttgtgtgcctgtttttctattttacgtaaatcaccctgaacatgtttgcatcaacctactggtgatgcacctttgatcaatacattttagacaaacgtggtttttgagtccaaagatcagggctgggttgacctgaatactggatacagggcatataaaacaggggcaaggcacagactcatagcagagcaatcaccaccaagcctggaataactgcaagggctctgctgacatcttcctgaggtgccaaggaaatgagg

SEQ ID NO: 11 - DNA, 2172 bp, Artificial Sequence
  Description of Artificial Sequence: wildtype GPE, but lacking Alu - 2 and Alu - 3
cctttgagaatccacggtgtctcgatgcagtcagctttctaacaagctggggcctcacctgttttcccacggataaaaacgtgctggaggaagcagaaaggggctggcaggtggaaagatgaggaccagctcatcgtctcatgactatgaggttgctctgatccagagggtccccctgcctggtggcccaccgccaggaagactcccactgtccctggatgcccagagtgggatgtcaactccatcacttatcaactccttatccataggggtattcttcctgaggcgtctcagaaaacagggccctccccatatgctgaccacataatagaacccctcccaactcagagaccctggctgctagctgccctggcatgacccagacagtggcctttgtatatgtttttagactcaccttgactcacctctgaccatagaaactctcatcccagaggtcactgcaatagttactccacaacagaggcttatctgggtagagggaggctccctacctatggcccagcagccctgacagtgcagatcacatataccccacgccccagcactgcctgccacgcatgggcttactttacacccacccacagtcaccaacacattacctgctctccaaggttaggcgtggcaggagaagtttgcttggaccagcagaaaccatgcagtcaaggacaactggagtcagcatgggctgggtgcgagcccttggtggggtggggaggagactccaggtcatacctcctggaggatgttttaatcatttccagcatggaatgctgtcaacttttgccacagattcattagctctgagtttcttttttctgtccccagctaccccttacatgtcaatatggacttaatgatgggaaattcaggcaagtttttaaacattttattccccctggctcttatcctcaaaaaatgcatgaatttggaggcagtggctcatgcctgtaatcccaatgctttgctaggttgaggcgggaggatcacttgaagccaggaatttgagaccagcctgggccgcatagtgagaccccgtttctacaaaaataaataaataaataataaataatagtgatatgaagcatgattaaatagccctattttttaaaatgcatgagttcgttacctgattcattccctggttcctttcacagtcctccgtgacccaagtgttagggttttggtctctctactatttgtaggctgatatatagtatacacacacacacacacacacatatacacacacacagtgtatcttgagctttcttttgtatatctacacacatatgtataagaaagctcaagatatagaagccctttttcaaaaataactgaaagtttcaaactctttaagtctccagttaccattttgctggtattcttatttggaaccatacattcatcatattgttgcacagtaagactatacattcattattttgcttaaacgtatgagttaaaacactttaaggtcattaaatgaattaatcactgcattcaaaaacgattactttctggccctaagagacatgaggccaataccaggaagggggttgatctcccaaaccagaggcagaccctagactctaatacagttaaggaaagaccagcaagatgatagtccccaatacaatagaactttactaattttaaaattaagaacttaaaacttgaatagctagagcaccaagatttttctttgtccccaaataagtgcagttgcaggcatagaaaatctgacatctttgcaagaatcatcgtggatgtagactctgtcctgtgtctctggcctggtttcggggaccaggagggcagacccttgcactgccaagaagcatgccaaagttaatcattggccctgctgagtacatggccgatcaggctgtttttgtgtgcctgtttttctattttacgtaaatcaccctgaacatgtttgcatcaacctactggtgatgcacctttgatcaatacattttagacaaacgtggtttttgagtccaaagatcagggctgggttgacctgaatactggatacagggcatataaaacaggggcaaggcacagactcatagcagagcaatcaccaccaagcctggaataactgcaagggctctgctgacatcttcctgaggtgccaaggaaatgagg

SEQ ID NO: 12 - DNA, 2314 bp, Artificial Sequence
  Description of Artificial Sequence: wildtype GPE, but lacking Alu - 1 and Alu - 3
cctttgagaatccacggtgtctcgatgcagtcagctttctaacaagctggggcctcacctgttttcccacggataaaaacgtgctggaggaagcagaaaggggctggcaggtggaaagatgaggaccagctcatcgtctcatgactatgaggttgctctgatccagagggtccccctgcctggtggcccaccgccaggaagactcccactgtccctggatgcccagagtgggatgtcaactccatcacttatcaactccttatccataggggtattcttcctgaggcgtctcagaaaacagggccctccccatatgctgaccacataatagaacccctcccaactcagagaccctggctgctagctgccctggcatgacccagacagtggcctttgtatatgtttttagactcaccttgactcacctctgaccatagaaactctcatcccagaggtcactgcaatagttactccacaacagaggcttatctgggtagagggaggctccctacctatggcccagcagccctgacagtgcagatcacatataccccacgccccagcactgcctgccacgcatgggcttactttacacccacccacagtcaccaacacattacctgctctccaaggttaggcgtggcaggagaagtttgcttggaccagcagaaaccatgcagtcaaggacaactggagtcagcatgggctgggtgcgagcccttggtggggtggggaggagactccaggtcatacctcctggaggatgttttaatcatttccagcatggaatgctgtcaacttttgccacagattcattagctctgagtttcttttttctgtccccagctaccccttacatgtcaatatggacttaatgatgggaaattcaggcaagtttttaaacattttattccccctggctcttatcctcaaaaaatgcatgagttcgttacctgattcattccctggttcctttcacagtcctccgtgacccaagtgttagggttttggtctctctactatttgtaggctgatatatagtatacacacacacacacacacacatatacacacacacagtgtatcttgagctttcttttgtatatctacacacatatgtataagaaagctcaagatatagaagccctttttcaaaaataactgaaagtttcaaactctttaagtctccagttaccattttgctggtattcttatttggaaccatacattcatcatattgttgcacagtaagactatacattcattattttgcttaaacgtatgagttaaaacacttggccaggcatggtggttcacacctgtaatcccagagctttgggaagccaagactggcagatctcttgagctcaggaattcaagaccagcctgggcaacatggaaaaaccccatctctacaaaagatagaaaaattagccaggcatggtggcgtgtgcctgtggtcccagctactcaggaggctgaggtgggaggatcacattagcccaggaggttgaggctgcagtgagccgtgattatgccactgcactccagcctgggagacagagtgagaccctgtttcaaaaaaaagagagagaaaatttaaaaaagaaaacaacaccaagggctgtaactttaaggtcattaaatgaattaatcactgcattcaaaaacgattactttctggccctaagagacatgaggccaataccaggaagggggttgatctcccaaaccagaggcagaccctagactctaatacagttaaggaaagaccagcaagatgatagtccccaatacaatagaactttactaattttaaaattaagaacttaaaacttgaatagctagagcaccaagatttttctttgtccccaaataagtgcagttgcaggcatagaaaatctgacatctttgcaagaatcatcgtggatgtagactctgtcctgtgtctctggcctggtttcggggaccaggagggcagacccttgcactgccaagaagcatgccaaagttaatcattggccctgctgagtacatggccgatcaggctgtttttgtgtgcctgtttttctattttacgtaaatcaccctgaacatgtttgcatcaacctactggtgatgcacctttgatcaatacattttagacaaacgtggtttttgagtccaaagatcagggctgggttgacctgaatactggatacagggcatataaaacaggggcaaggcacagactcatagcagagcaatcaccaccaagcctggaataactgcaagggctctgctgacatcttcctgaggtgccaaggaaatgagg

SEQ ID NO: 13 - DNA, 301 bp, Artificial Sequence
  Description of Artificial Sequence: Intron
agctttattgcggtagtttatcacagttaaattgctaacgcagtcagtgcttctgacacaacagtctcgaacttaagctgcagtgactctcttaaggtagccttgcagaagttggtcgtgaggcactgggcaggtaagtatcaaggttacaagacaggtttaaggagaccaatagaaactgggcttgtcgagacagagaagactcttgcgtttctgataggcacctattggtcttactgacatccactttgcctttctctccacaggtgtccactcccagttcaattacagctcttaaggc

SEQ ID NO: 14 - DNA, 137 bp, Artificial Sequence
  Description of Artificial Sequence: SV40 polyA tail
ggccgctatttgtgaaatttgtgatgctattgctttatttgtaaccattataagctgcaataaacaagttaacaacaacaattgcattcattttatgtttcaggttcagggggaggtgtgggaggttttttaggcat

SEQ ID NO: 15 - DNA, 145 bp, Artificial Sequence
  Description of Artificial Sequence: AAV2 ITR
ttggccactccctctctgcgcgctcgctcgctcactgaggccgggcgaccaaaggtcgcccgacgcccgggctttgcccgggcggcctcagtgagcgagcgagcgcgcagagagggagtggccaactccatcactaggggttcct